European Patent Application EP 4 361 257 A1, published May 1, 2024. Title: ONCOLYTIC VIRUS AND USE THEREOF. Applicant: JOINT BIOSCIENCES (SH) LTD. The sequence listing filed with the application follows.

SEQUENCE LISTING (28 sequences)

SEQ ID NO: 1 - protein, 229 aa, unidentified
  source 1..229: note = Indiana strain MuddSummer subtype of vesicular stomatitis virus
MSSLKKILGLKGKGKKSKKLGIAPPPYEEDTNMEYAPSAPIDKSYFGVDEMDTHDPNQLRYEKFFFTVKMTVRSNRPFRTYSDVAAAVSHWDHMYIGMAGKRPFYKILAFLGSSNLKATPAVLADQGQPEYHAHCEGRAYLPHRMGKTPPMLNVPEHFRRPFNIGLYKGTIELTMTIYDDESLEAAPMIWDHFNSSKFSDFREKALMFGLIVEKKASGAWVLDSVSHFK

SEQ ID NO: 2 - protein, 511 aa, unidentified
  source 1..511: note = Indiana strain MuddSummer subtype of vesicular stomatitis virus
MKCLLYLAFLFIGVNCKFTIVFPHNQKGNWKNVPSNYHYCPSSSDLNWHNDLVGTALQVKMPKSHKAIQADGWMCHASKWVTTCDFRWYGPKYITHSIRSFTPSVEQCKESIEQTKQGTWLNPGFPPQSCGYATVTDAEAAIVQVTPHHVLVDEYTGEWVDSQFINGKCSNDICPTVHNSTTWHSDYKVKGLCDSNLISMDITFFSEDGELSSLGKKGTGFRSNYFAYETGDKACKMQYCKHWGVRLPSGVWFEMADKDLFAAARFPECPEGSSISAPSQTSVDVSLIQDVERILDYSLCQETWSKIRAGLPISPVDLSYLAPKNPGTGPVFTIINGTLKYFETRYIRVDIAAPILSRMVGMISGTTTERVLWDDWAPYEDVEIGPNGVLRTSSGYKFPLYMIGHGMLDSDLHLSSKAQVFEHPHIQDAASQLPDGETLFFGDTGLSKNPIEFVEGWFSSWKSSIASFFFTIGLIIGLFLVLRVGIYLCIKLKHTKKRQIYTDIEMNRLGK

SEQ ID NO: 3 - protein, 229 aa, synthetic construct
MSSLKKILGLKGKGKKSKKLGIAPPPYEEDTSMEYAPSAPIDKSYFGVDERDTYDPNQLRYEKFFFTVKMTVRSNRPFRTYSDVAAAVSHWDHMYIGMAGKRPFYKILAFLGSSNLKATPAVLADQGQPEYHAHCEGRAYLPHRMGKTPPMLNVPEHFRRPFNIGLYKGTIELTMTIYDDESLEAAPMIWDHFNSSKFSDFREKALMFGLIVEKKASGAWVLDSISHFK

SEQ ID NO: 4 - protein, 229 aa, synthetic construct
MSSLKKILGLKGKGKKSKKLGIAPPPYEEDTSMEYAPSAPIDKSYFGVDERDTYDPNQLRYEKFFFTVKMTVRSNRPFRTYSDVAAAVSHWDHMYIGMAGKRPFYKILAFLGSSNLKATPAVLADQGQPEYHAHCEGRAYLPHRMGKTPPMLNVPEHFRRPFNIGLYKGTIELTMTIYDDESLEAAPMIWDHFNSSKFSDFREKALMFGLIVEKKASGAWFLDSISHFK

SEQ ID NO: 5 - protein, 229 aa, synthetic construct
MSSLKKILGLKGKGKKSKKLGIAPPPYEEDTSMEYAPSAPIDKSYFGVDERDTYDPNQLRYEKFFFTVKMTVRSNRPFRTYSDVAAAVSHWDHMYIGMAGKRPFYKILAFLGSSNLKATPAVLADQGQPEYHAHCEGRAYLPHRMGKTPPMLNVPEHFRRPFNIGLYKGTIELTMTIYDDESLEAAPMIWDHFNSSKFSDFREKALMFGLIVEKKASGAWFLDSIRHFK

SEQ ID NO: 6 - protein, 511 aa, unidentified
MKCLLYLAFLFIGVNCKFTIVFPHNQKGNWKNVPSNYHYCPSSSDLNWHNDLIGTALQVKMPKSHKAIQADGWMCHASKWVTTCDFRWYGPKYITHSIRSFTPSVEQCKESIEQTKQGTWLNPGFPPQSCGYATVTDAEAAIVQVTPHHVLVDEYTGEWVDSQFINGKCSNDICPTVHNSTTWHSDYKVKGLCDSNLISMDITFFSEDGELSSLGKKGTGFRSNYFAYETGDKACKMQYCKHWGVRLPSGVWFEMADKDLFAAARFPECPEGSSISAPSQTSVDVSLIQDVERILDYSLCQETWSKIRAGLPISPVDLSYLAPKNPGTGPVFTIINGTLKYFETRYIRVDIAAPILSRMVGMISGTTTERVLWDDWAPYEDVEIGPNGVLRTSSGYKFPLYMIGHGMLDSDLHLSSKAQVFEHPHIQDAASQLPDGETLFFGDTGLSKNPIEFVEGWFSSWKSSIASFFFTIGLIIGLFLVLRVGIYLCIKLKHTKKRQIYTDIEMNRLGK

SEQ ID NO: 7 - protein, 511 aa, synthetic construct
MKCLLYLAFLFIGVNCKFTIVFPHNQKGNWKNVPSNYHYCPSSSDLNWHNDLIGTALQVKMPKSHKAIQADGWMCHASKWVTTCDFRWYGPKYITHSIRSFTPSVEQCKESIEQTKQGTWLNPGFPPQSCGYATVTDAEAVIVQVTPHHVLVDEYTGEWVDSQFINGKCSNDICPTVHNSTTWHSDYKVKGLCDSNLISMDITFFSEDGELSSLGKKGTGFRSNYFAYETGDKACKMQYCKHWGVRLPSGVWFEMADKDLFAAARFPECPEGSSISAPSQTSVDVSLIQDVERILDYSLCQETWSKIRAGLPISPVDLSYLAPKNPGTGPVFTIINGTLKYFETRYIRVDIAAPILSRMVGMISGTTTERVLWDDWAPYEDVEIGPNGVLRTSSGYKFPLYMIGHGMLDSDLHLSSKAQVFEHPHIQDAASQLPDGETLFFGDTGLSKNPIEFVEGWFSSWKSSIASFFFTIGLIIGLFLVLRVGIYLCIKLKHTKKRQIYTDIEMNRLGK

SEQ ID NO: 8 - protein, 511 aa, synthetic construct
MKCLLYLAFLFIGVNCKFTIVFPHNQKGNWKNVPSNYHYCPSSSDLNWHNDLIGTALQVKMPKSHKAIQADGWMCHASKWVTTCDFRWYGPKYITHSIRSFTPSVEQCKESIEQTKQGTWLNPGFPPQSCGYATVTDAEAVIVQVTPHHVLVDEYTGEWVDSQFINGKCSNYICPTVHNSTTWHSDYKVKGLCDSNLISMDITFFSEDGELSSLGKKGTGFRSNYFAYETGDKACKMQYCKHWGVRLPSGVWFEMADKDLFAAARFPECPEGSSISAPSQTSVDVSLIQDVERILDYSLCQETWSKIRAGLPISPVDLSYLAPKNPGTGPVFTIINGTLKYFETRYIRVDIAAPILSRMVGMISGTTTERVLWDDWAPYEDVEIGPNGVLRTSSGYKFPLYMIGHGMLDSDLHLSSKAQVFEHPHIQDAASQLPDGETLFFGDTGLSKNPIEFVEGWFSSWKSSIASFFFTIGLIIGLFLVLRVGIYLCIKLKHTKKRQIYTDIEMNRLGK

SEQ ID NO: 9 - protein, 511 aa, synthetic construct
MKCLLYLAFLFIGVNCKFTIVFPHNQKGNWKNVPSNYHYCPSSSDLNWHNDLIGTALQVKMPKSHKAIQADGWMCHASKWVTTCDFRWYGPKYITHSIRSFTPSVEQCKESIEQTKQGTWLNPGFPPQSCGYATVTDAEAVIVQVTPHHVLVDEYTGEWVDSQFINGKCSNYICPTVHNSTTWHSDYKVKGLCDSNLISMDITFFSEDGELSSLGKEGTGFRSNYFAYETGDKACKMQYCKHWGVRLPSGVWFEMADKDLFAAARFPECPEGSSISAPSQTSVDVSLIQDVERILDYSLCQETWSKIRAGLPISPVDLSYLAPKNPGTGPVFTIINGTLKYFETRYIRVDIAAPILSRMVGMISGTTTERVLWDDWAPYEDVEIGPNGVLRTSSGYKFPLYMIGHGMLDSDLHLSSKAQVFEHPHIQDAASQLPDGETLFFGDTGLSKNPIEFVEGWFSSWKSSIASFFFTIGLIIGLFLVLRVGIYLCIKLKHTKKRQIYTDIEMNRLGK

SEQ ID NO: 10 - protein, 511 aa, synthetic construct
MKCLLYLAFLFIGVNCKFTIVFPHNQKGNWKNVPSNYHYCPSSSDLNWHNDLIGTALQVKMPKSHKAIQADGWMCHASKWVTTCDFRWYGPKYITHSIRSFTPSVEQCKESIEQTKQGTWLNPGFPPQSCGYATVTDAEAVIVQVTPHHVLVDEYTGEWVDSQFINGKCSNYICPTVHNSTTWHSDYKVKGLCDSNLISMDITFFSEDGELSSLGKEGTGFRSNYFAYETGGKACKMQYCKHWGVRLPSGVWFEMADKDLFAAARFPECPEGSSISAPSQTSVDVSLIQDVERILDYSLCQETWSKIRAGLPISPVDLSYLAPKNPGTGPVFTIINGTLKYFETRYIRVDIAAPILSRMVGMISGTTTERVLWDDWAPYEDVEIGPNGVLRTSSGYKFPLYMIGHGMLDSDLHLSSKAQVFEHPHIQDAASQLPDGETLFFGDTGLSKNPIEFVEGWFSSWKSSIASFFFTIGLIIGLFLVLRVGIYLCIKLKHTKKRQIYTDIEMNRLGK

SEQ ID NO: 11 - protein, 511 aa, synthetic construct
MKCLLYLAFLFIGVNCKFTIVFPHNQKGNWKNVPSNYHYCPSSSDLNWHNDLIGTALQVKMPKSHKAIQADGWMCHASKWVTTCDFRWYGPKYITHSIRSFTPSVEQCKESIEQTKQGTWLNPGFPPQSCGYATVTDAEAVIVQVTPHHVLVDEYTGEWVDSQFINGKCSNYICPTVHNSTTWHSDYKVKGLCDSNLISMDITFFSEDGELSSLGKEGTGFRSNYFAYETGGKACKMQYCKHWGVRLPSGVWFEMADKDLFAAARFPECPEGSSISAPSQTSVDVSLIQDVERILDYSLCQETWSKIRAGLPISPVDLSYLAPKNPGTGPAFTIINGTLKYFETRYIRVDIAAPILSRMVGMISGTTTERVLWDDWAPYEDVEIGPNGVLRTSSGYKFPLYMIGHGMLDSDLHLSSKAQVFEHPHIQDAASQLPDGETLFFGDTGLSKNPIEFVEGWFSSWKSSIASFFFTIGLIIGLFLVLRVGIYLCIKLKHTKKRQIYTDIEMNRLGK

SEQ ID NO: 12 - protein, 511 aa, synthetic construct
MKCLLYLAFLFIGVNCKFTIVFPHNQKGNWKNVPSNYHYCPSSSDLNWHNDLIGTALQVKMPKSHKAIQADGWMCHASKWVTTCDFRWYGPKYITHSIRSFTPSVEQCKESIEQTKQGTWLNPGFPPQSCGYATVTDAEAVIVQVTPHHVLVDEYTGEWVDSQFINGKCSNYICPTVHNSTTWHSDYKVKGLCDSNLISMDITFFSEDGELSSLGKEGTGFRSNYFAYETGGKACKMQYCKHWGVRLPSGVWFEMADKDLFAAARFPECPEGSSISAPSQTSVDVSLIQDVERILDYSLCQETWSKIRAGLPISPVDLSYLAPKNPGTGPAFTIINGTLKYFETRYIRVDIAAPILSRMVGMISGTTTERELWDDWAPYEDVEIGPNGVLRTSSGYKFPLYMIGHGMLDSDLHLSSKAQVFEHPHIQDAASQLPDGETLFFGDTGLSKNPIEFVEGWFSSWKSSIASFFFTIGLIIGLFLVLRVGIYLCIKLKHTKKRQIYTDIEMNRLGK

SEQ ID NO: 13 - protein, 511 aa, synthetic construct
MKCLLYLAFLFIGVNCKFTIVFPHNQKGNWKNVPSNYHYCPSSSDLNWHNDLIGTALQVKMPKSHKAIQADGWMCHASKWVTTCDFRWYGPKYITHSIRSFTPSVEQCKESIEQTKQGTWLNPGFPPQSCGYATVTDAEAVIVQVTPHHVLVDEYTGEWVDSQFINGKCSNYICPTVHNSTTWHSDYKVKGLCDSNLISMDITFFSEDGELSSLGKEGTGFRSNYFAYETGGKACKMQYCKHWGVRLPSGVWFEMADKDLFAAARFPECPEGSSISAPSQTSVDVSLIQDVERILDYSLCQETWSKIRAGLPISPVDLSYLAPKNPGTGPAFTIINGTLKYFETRYIRVDIAAPILSRMVGMISGTTTERELWDDWAPYEDVEIGPNGVLRTSSGYKFPLYMIGHGMLDSDLHLSSKAQVFEHPHIQDAASQLPDDETLFFGDTGLSKNPIEFVEGWFSSWKSSIASFFFTIGLIIGLFLVLRVGIYLCIKLKHTKKRQIYTDIEMNRLGK

SEQ ID NO: 14 - protein, 511 aa, synthetic construct
MKCLLYLAFLFIGVNCKFTIVFPHNQKGNWKNVPSNYHYCPSSSDLNWHNDLIGTALQVKMPKSHKAIQADGWMCHASKWVTTCDFRWYGPKYITHSIRSFTPSVEQCKESIEQTKQGTWLNPGFPPQSCGYATVTDAEAVIVQVTPHHVLVDEYTGEWVDSQFINGKCSNYICPTVHNSTTWHSDYKVKGLCDSNLISMDITFFSEDGELSSLGKEGTGFRSNYFAYETGGKACKMQYCKHWGVRLPSGVWFEMADKDLFAAARFPECPEGSSISAPSQTSVDVSLIQDVERILDYSLCQETWSKIRAGLPISPVDLSYLAPKNPGTGPAFTIINGTLKYFETRYIRVDIAAPILSRMVGMISGTTTERELWDDWAPYEDVEIGPNGVLRTSSGYKFPLYMIGHGMLDSDLHLSSKAQVFEHPHIQDAASQLPDDESLFFGDTGLSKNPIEFVEGWFSSWKSSIASFFFTIGLIIGLFLVLRVGIYLCIKLKHTKKRQIYTDIEMNRLGK

SEQ ID NO: 15 - protein, 511 aa, synthetic construct
MKCLLYLAFLFIGVNCKFTIVFPHNQKGNWKNVPSNYHYCPSSSDLNWHNDLIGTALQVKMPKSHKAIQADGWMCHASKWVTTCDFRWYGPKYITHSIRSFTPSVEQCKESIEQTKQGTWLNPGFPPQSCGYATVTDAEAVIVQVTPHHVLVDEYTGEWVDSQFINGKCSNYICPTVHNSTTWHSDYKVKGLCDSNLISMDITFFSEDGELSSLGKEGTGFRSNYFAYETGGKACKMQYCKHWGVRLPSGVWFEMADKDLFAAARFPECPEGSSISAPSQTSVDVSLIQDVERILDYSLCQETWSKIRAGLPISPVDLSYLAPKNPGTGPAFTIINGTLKYFETRYIRVDIAAPILSRMVGMISGTTTERELWDDWAPYEDVEIGPNGVLRTSSGYKFPLYMIGHGMLDSDLHLSSKAQVFEHPHIQDAASQLPDDESLFFGDTGLSKNPIELVEGWFSSWKSSIASFFFTIGLIIGLFLVLRVGIYLCIKLKHTKKRQIYTDIEMNRLGK

SEQ ID NO: 16 - protein, 511 aa, synthetic construct
MKCLLYLAFLFIGVNCKFTIVFPHNQKGNWKNVPSNYHYCPSSSDLNWHNDLIGTALQVKMPKSHKAIQADGWMCHASKWVTTCDFRWYGPKYITHSIRSFTPSVEQCKESIEQTKQGTWLNPGFPPQSCGYATVTDAEAVIVQVTPHHVLVDEYTGEWVDSQFINGKCSNYICPTVHNSTTWHSDYKVKGLCDSNLISMDITFFSEDGELSSLGKEGTGFRSNYFAYETGGKACKMQYCKHWGVRLPSGVWFEMADKDLFAAARFPECPEGSSISAPSQTSVDVSLIQDVERILDYSLCQETWSKIRAGLPISPVDLSYLAPKNPGTGPAFTIINGTLKYFETRYIRVDIAAPILSRMVGMISGTTTERELWDDWAPYEDVEIGPNGVLRTSSGYKFPLYMIGHGMLDSDLHLSSKAQVFEHPHIQDAASQLPDDESLFFGDTGLSKNPIELVEGWFSSWKSSIASFFFIIGLIIGLFLVLRVGIYLCIKLKHTKKRQIYTDIEMNRLGK

SEQ ID NO: 17 - protein, 511 aa, synthetic construct
MKCLLYLAFLFIGVNCKFTIVFPHNQKGNWKNVPSNYHYCPSSSDLNWHNDLIGTALQVKMPKSHKAIQADGWMCHASKWVTTCDFRWYGPKYITHSIRSFTPSVEQCKESIEQTKQGTWLNPGFPPQSCGYATVTDAEAVIVQVTPHHVLVDEYTGEWVDSQFINGKCSNYICPTVHNSTTWHSDYKVKGLCDSNLISMDITFFSEDGELSSLGKEGTGFRSNYFAYETGGKACKMQYCKHWGVRLPSGVWFEMADKDLFAAARFPECPEGSSISAPSQTSVDVSLIQDVERILDYSLCQETWSKIRAGLPISPVDLSYLAPKNPGTGPAFTIINGTLKYFETRYIRVDIAAPILSRMVGMISGTTTERELWDDWAPYEDVEIGPNGVLRTSSGYKFPLYMIGHGMLDSDLHLSSKAQVFEHPHIQDAASQLPDDESLFFGDTGLSKNPIELVEGWFSSWKSSIASFFFIIGLIIGLFLVLRVGIHLCIKLKHTKKRQIYTDIEMNRLGK

SEQ ID NO: 18 - protein, 511 aa, synthetic construct
MKCLLYLAFLFIGVNCKFTIVFPHNQKGNWKNVPSNYHYCPSSSDLNWHNDLVGTALQVKMPKSHKAIQADGWMCHASKWVTTCDFRWYGPKYITHSIRSFTPSVEQCKESIEQTKQGTWLNPGFPPQSCGYATVTDAEAVIVQVTPHHVLVDEYTGEWVDSQFINGKCSNYICPTVHNSTTWHSDYKVKGLCDSNLISMDITFFSEDGELSSLGKEGTGFRSNYFAYETGGKACKMQYCKHWGVRLPSGVWFEMADKDLFAAARFPECPEGSSISAPSQTSVDVSLIQDVERILDYSLCQETWSKIRAGLPISPVDLSYLAPKNPGTGPAFTIINGTLKYFETRYIRVDIAAPILSRMVGMISGTTTERELWDDWAPYEDVEIGPNGVLRTSSGYKFPLYMIGHGMLDSDLHLSSKAQVFEHPHIQDAASQLPDDESLFFGDTGLSKNPIELVEGWFSSWKSSIASFFFIIGLIIGLFLVLRVGIHLCIKLKHTKKRQIYTDIEMNRLGK

SEQ ID NO: 19 - protein, 511 aa, synthetic construct
MKCLLYLAFLFIGVNCKFTIVFPHNQKGNWKNVPSNYHYCPSSSDLNWHNDLVGTALQVKMPKSHKAIQADGWMCHASKWVTTCDFRWYGPKYITHSIRSFTPSVEQCKESIEQTKQGTWLNPGFPPQSCGYATVTDAEAAIVQVTPHHVLVDEYTGEWVDSQFINGKCSNYICPTVHNSTTWHSDYKVKGLCDSNLISMDITFFSEDGELSSLGKEGTGFRSNYFAYETGGKACKMQYCKHWGVRLPSGVWFEMADKDLFAAARFPECPEGSSISAPSQTSVDVSLIQDVERILDYSLCQETWSKIRAGLPISPVDLSYLAPKNPGTGPAFTIINGTLKYFETRYIRVDIAAPILSRMVGMISGTTTERELWDDWAPYEDVEIGPNGVLRTSSGYKFPLYMIGHGMLDSDLHLSSKAQVFEHPHIQDAASQLPDDESLFFGDTGLSKNPIELVEGWFSSWKSSIASFFFIIGLIIGLFLVLRVGIHLCIKLKHTKKRQIYTDIEMNRLGK

SEQ ID NO: 20 - protein, 511 aa, synthetic construct
MKCLLYLAFLFIGVNCKFTIVFPHNQKGNWKNVPSNYHYCPSSSDLNWHNDLVGTALQVKMPKSHKAIQADGWMCHASKWVTTCDFRWYGPKYITHSIRSFTPSVEQCKESIEQTKQGTWLNPGFPPQSCGYATVTDAEAAIVQVTPHHVLVDEYTGEWVDSQFINGKCSNDICPTVHNSTTWHSDYKVKGLCDSNLISMDITFFSEDGELSSLGKEGTGFRSNYFAYETGGKACKMQYCKHWGVRLPSGVWFEMADKDLFAAARFPECPEGSSISAPSQTSVDVSLIQDVERILDYSLCQETWSKIRAGLPISPVDLSYLAPKNPGTGPAFTIINGTLKYFETRYIRVDIAAPILSRMVGMISGTTTERELWDDWAPYEDVEIGPNGVLRTSSGYKFPLYMIGHGMLDSDLHLSSKAQVFEHPHIQDAASQLPDDESLFFGDTGLSKNPIELVEGWFSSWKSSIASFFFIIGLIIGLFLVLRVGIHLCIKLKHTKKRQIYTDIEMNRLGK

SEQ ID NO: 21 - protein, 511 aa, synthetic construct
MKCLLYLAFLFIGVNCKFTIVFPHNQKGNWKNVPSNYHYCPSSSDLNWHNDLVGTALQVKMPKSHKAIQADGWMCHASKWVTTCDFRWYGPKYITHSIRSFTPSVEQCKESIEQTKQGTWLNPGFPPQSCGYATVTDAEAAIVQVTPHHVLVDEYTGEWVDSQFINGKCSNDICPTVHNSTTWHSDYKVKGLCDSNLISMDITFFSEDGELSSLGKKGTGFRSNYFAYETGGKACKMQYCKHWGVRLPSGVWFEMADKDLFAAARFPECPEGSSISAPSQTSVDVSLIQDVERILDYSLCQETWSKIRAGLPISPVDLSYLAPKNPGTGPAFTIINGTLKYFETRYIRVDIAAPILSRMVGMISGTTTERELWDDWAPYEDVEIGPNGVLRTSSGYKFPLYMIGHGMLDSDLHLSSKAQVFEHPHIQDAASQLPDDESLFFGDTGLSKNPIELVEGWFSSWKSSIASFFFIIGLIIGLFLVLRVGIHLCIKLKHTKKRQIYTDIEMNRLGK

SEQ ID NO: 22 - protein, 511 aa, synthetic construct
MKCLLYLAFLFIGVNCKFTIVFPHNQKGNWKNVPSNYHYCPSSSDLNWHNDLVGTALQVKMPKSHKAIQADGWMCHASKWVTTCDFRWYGPKYITHSIRSFTPSVEQCKESIEQTKQGTWLNPGFPPQSCGYATVTDAEAAIVQVTPHHVLVDEYTGEWVDSQFINGKCSNDICPTVHNSTTWHSDYKVKGLCDSNLISMDITFFSEDGELSSLGKKGTGFRSNYFAYETGDKACKMQYCKHWGVRLPSGVWFEMADKDLFAAARFPECPEGSSISAPSQTSVDVSLIQDVERILDYSLCQETWSKIRAGLPISPVDLSYLAPKNPGTGPAFTIINGTLKYFETRYIRVDIAAPILSRMVGMISGTTTERELWDDWAPYEDVEIGPNGVLRTSSGYKFPLYMIGHGMLDSDLHLSSKAQVFEHPHIQDAASQLPDDESLFFGDTGLSKNPIELVEGWFSSWKSSIASFFFIIGLIIGLFLVLRVGIHLCIKLKHTKKRQIYTDIEMNRLGK

SEQ ID NO: 23 - protein, 511 aa, synthetic construct
MKCLLYLAFLFIGVNCKFTIVFPHNQKGNWKNVPSNYHYCPSSSDLNWHNDLVGTALQVKMPKSHKAIQADGWMCHASKWVTTCDFRWYGPKYITHSIRSFTPSVEQCKESIEQTKQGTWLNPGFPPQSCGYATVTDAEAAIVQVTPHHVLVDEYTGEWVDSQFINGKCSNDICPTVHNSTTWHSDYKVKGLCDSNLISMDITFFSEDGELSSLGKKGTGFRSNYFAYETGDKACKMQYCKHWGVRLPSGVWFEMADKDLFAAARFPECPEGSSISAPSQTSVDVSLIQDVERILDYSLCQETWSKIRAGLPISPVDLSYLAPKNPGTGPVFTIINGTLKYFETRYIRVDIAAPILSRMVGMISGTTTERELWDDWAPYEDVEIGPNGVLRTSSGYKFPLYMIGHGMLDSDLHLSSKAQVFEHPHIQDAASQLPDDESLFFGDTGLSKNPIELVEGWFSSWKSSIASFFFIIGLIIGLFLVLRVGIHLCIKLKHTKKRQIYTDIEMNRLGK

SEQ ID NO: 24 - protein, 511 aa, synthetic construct
MKCLLYLAFLFIGVNCKFTIVFPHNQKGNWKNVPSNYHYCPSSSDLNWHNDLVGTALQVKMPKSHKAIQADGWMCHASKWVTTCDFRWYGPKYITHSIRSFTPSVEQCKESIEQTKQGTWLNPGFPPQSCGYATVTDAEAAIVQVTPHHVLVDEYTGEWVDSQFINGKCSNDICPTVHNSTTWHSDYKVKGLCDSNLISMDITFFSEDGELSSLGKKGTGFRSNYFAYETGDKACKMQYCKHWGVRLPSGVWFEMADKDLFAAARFPECPEGSSISAPSQTSVDVSLIQDVERILDYSLCQETWSKIRAGLPISPVDLSYLAPKNPGTGPVFTIINGTLKYFETRYIRVDIAAPILSRMVGMISGTTTERVLWDDWAPYEDVEIGPNGVLRTSSGYKFPLYMIGHGMLDSDLHLSSKAQVFEHPHIQDAASQLPDDESLFFGDTGLSKNPIELVEGWFSSWKSSIASFFFIIGLIIGLFLVLRVGIHLCIKLKHTKKRQIYTDIEMNRLGK

SEQ ID NO: 25 - protein, 511 aa, synthetic construct
MKCLLYLAFLFIGVNCKFTIVFPHNQKGNWKNVPSNYHYCPSSSDLNWHNDLVGTALQVKMPKSHKAIQADGWMCHASKWVTTCDFRWYGPKYITHSIRSFTPSVEQCKESIEQTKQGTWLNPGFPPQSCGYATVTDAEAAIVQVTPHHVLVDEYTGEWVDSQFINGKCSNDICPTVHNSTTWHSDYKVKGLCDSNLISMDITFFSEDGELSSLGKKGTGFRSNYFAYETGDKACKMQYCKHWGVRLPSGVWFEMADKDLFAAARFPECPEGSSISAPSQTSVDVSLIQDVERILDYSLCQETWSKIRAGLPISPVDLSYLAPKNPGTGPVFTIINGTLKYFETRYIRVDIAAPILSRMVGMISGTTTERVLWDDWAPYEDVEIGPNGVLRTSSGYKFPLYMIGHGMLDSDLHLSSKAQVFEHPHIQDAASQLPDGESLFFGDTGLSKNPIELVEGWFSSWKSSIASFFFIIGLIIGLFLVLRVGIHLCIKLKHTKKRQIYTDIEMNRLGK

SEQ ID NO: 26 - protein, 511 aa, synthetic construct
MKCLLYLAFLFIGVNCKFTIVFPHNQKGNWKNVPSNYHYCPSSSDLNWHNDLVGTALQVKMPKSHKAIQADGWMCHASKWVTTCDFRWYGPKYITHSIRSFTPSVEQCKESIEQTKQGTWLNPGFPPQSCGYATVTDAEAAIVQVTPHHVLVDEYTGEWVDSQFINGKCSNDICPTVHNSTTWHSDYKVKGLCDSNLISMDITFFSEDGELSSLGKKGTGFRSNYFAYETGDKACKMQYCKHWGVRLPSGVWFEMADKDLFAAARFPECPEGSSISAPSQTSVDVSLIQDVERILDYSLCQETWSKIRAGLPISPVDLSYLAPKNPGTGPVFTIINGTLKYFETRYIRVDIAAPILSRMVGMISGTTTERVLWDDWAPYEDVEIGPNGVLRTSSGYKFPLYMIGHGMLDSDLHLSSKAQVFEHPHIQDAASQLPDGETLFFGDTGLSKNPIELVEGWFSSWKSSIASFFFIIGLIIGLFLVLRVGIHLCIKLKHTKKRQIYTDIEMNRLGK

SEQ ID NO: 27 - protein, 511 aa, synthetic construct
MKCLLYLAFLFIGVNCKFTIVFPHNQKGNWKNVPSNYHYCPSSSDLNWHNDLVGTALQVKMPKSHKAIQADGWMCHASKWVTTCDFRWYGPKYITHSIRSFTPSVEQCKESIEQTKQGTWLNPGFPPQSCGYATVTDAEAAIVQVTPHHVLVDEYTGEWVDSQFINGKCSNDICPTVHNSTTWHSDYKVKGLCDSNLISMDITFFSEDGELSSLGKKGTGFRSNYFAYETGDKACKMQYCKHWGVRLPSGVWFEMADKDLFAAARFPECPEGSSISAPSQTSVDVSLIQDVERILDYSLCQETWSKIRAGLPISPVDLSYLAPKNPGTGPVFTIINGTLKYFETRYIRVDIAAPILSRMVGMISGTTTERVLWDDWAPYEDVEIGPNGVLRTSSGYKFPLYMIGHGMLDSDLHLSSKAQVFEHPHIQDAASQLPDGETLFFGDTGLSKNPIEFVEGWFSSWKSSIASFFFIIGLIIGLFLVLRVGIHLCIKLKHTKKRQIYTDIEMNRLGK

SEQ ID NO: 28 - protein, 480 aa, synthetic construct
MKCLLYLAFLFIGVNCKFTIVFPHNQKGNWKNVPSNYHYCPSSSDLNWHNDLVGTALQVKMPKSHKAIQADGWMCHASKWVTTCDFRWYGPKYITHSIRSFTPSVEQCKESIEQTKQGTWLNPGFPPQSCGYATVTDAEAAIVQVTPHHVLVDEYTGEWVDSQFINGKCSNDICPTVHNSTTWHSDYKVKGLCDSNLISMDITFFSEDGELSSLGKKGTGFRSNYFAYETGDKACKMQYCKHWGVRLPSGVWFEMADKDLFAAARFPECPEGSSISAPSQTSVDVSLIQDVERILDYSLCQETWSKIRAGLPISPVDLSYLAPKNPGTGPVFTIINGTLKYFETRYIRVDIAAPILSRMVGMISGTTTERVLWDDWAPYEDVEIGPNGVLRTSSGYKFPLYMIGHGMLDSDLHLSSKAQVFEHPHIQDAASQLPDGETLFFGDTGLSKNPIEFVEGWFSSWKSSIASFFFTIGLIIGLFL